European Patent Specification EP 3 651 786 B1, published October 25, 2023. Title: ANTIMICROBIAL PEPTIDES. Applicant: MATERIAS S.r.l. The sequence listing filed with the application follows.

SEQUENCE LISTING (4 sequences)

SEQ ID NO: 1 - protein, 12 aa, Unknown
  synthetic
VRLIVAVRIWRR

SEQ ID NO: 2 - protein, 12 aa, Unknown
  synthetic
VRLIVAVRIKRR

SEQ ID NO: 3 - protein, 12 aa, Unknown
  synthetic
VRLIVKVRIWRR

SEQ ID NO: 4 - protein, 12 aa, Unknown
  synthetic
VRLIVKVRIKRR